European Patent Application EP 4 414 457 A1, published August 14, 2024. Title: Method for analyzing structural variation, primer pair set and method for designing primer pair set. Applicant: 国立大学法人　東京大学. The sequence listing filed with the application follows.

SEQUENCE LISTING (30 sequences)

SEQ ID NO: 1 - DNA, 24 bp, synthetic construct
  source 1..24: mol_type = other DNA
ttttgatgggactagtggactttg

SEQ ID NO: 2 - DNA, 23 bp, synthetic construct
  source 1..23: mol_type = other DNA
aactgctcctaacccaccttgtc

SEQ ID NO: 3 - DNA, 24 bp, synthetic construct
  source 1..24: mol_type = other DNA
ttttgatgggactagtggactttg

SEQ ID NO: 4 - DNA, 23 bp, synthetic construct
  source 1..23: mol_type = other DNA
tcttgatctcctgacctcgtgat

SEQ ID NO: 5 - DNA, 18 bp, synthetic construct
  source 1..18: mol_type = other DNA
cagaaggaagagctatgc

SEQ ID NO: 6 - DNA, 15 bp, synthetic construct
  source 1..15: mol_type = other DNA
cagaaggcggtggct

SEQ ID NO: 7 - DNA, 25 bp, synthetic construct
  source 1..25: mol_type = other DNA
agtcttgctatggtgtctaagctgg

SEQ ID NO: 8 - DNA, 19 bp, synthetic construct
  source 1..19: mol_type = other DNA
cgcaagggagctcaatcct

SEQ ID NO: 9 - DNA, 25 bp, synthetic construct
  source 1..25: mol_type = other DNA
agtcttgctatggtgtctaagctgg

SEQ ID NO: 10 - DNA, 23 bp, synthetic construct
  source 1..23: mol_type = other DNA
gggccaaaaacatactcatcatg

SEQ ID NO: 11 - DNA, 36 bp, synthetic construct
  source 1..36: mol_type = other DNA
atactcctgcctcaacctcccaaagtgttaagatta

SEQ ID NO: 12 - DNA, 32 bp, synthetic construct
  source 1..32: mol_type = other DNA
cttgaactcttgtgaaaccaactggatcctga

SEQ ID NO: 13 - DNA, 24 bp, synthetic construct
  source 1..24: mol_type = other DNA
tcaatttaaaaagcctgcctatca

SEQ ID NO: 14 - DNA, 19 bp, synthetic construct
  source 1..19: mol_type = other DNA
aaagggtgcatcctggagg

SEQ ID NO: 15 - DNA, 24 bp, synthetic construct
  source 1..24: mol_type = other DNA
tcaatttaaaaagcctgcctatca

SEQ ID NO: 16 - DNA, 25 bp, synthetic construct
  source 1..25: mol_type = other DNA
ccatggaacttaccaagcactagtc

SEQ ID NO: 17 - DNA, 37 bp, synthetic construct
  source 1..37: mol_type = other DNA
aaagctttcttaggatgttgatttttgaatgtgcttt

SEQ ID NO: 18 - DNA, 31 bp, synthetic construct
  source 1..31: mol_type = other DNA
tgccttatgactcaagatgggagtttccaag

SEQ ID NO: 19 - DNA, 29 bp, synthetic construct
  source 1..29: mol_type = other DNA
aaatgagatcaatcagtacacgatatctg

SEQ ID NO: 20 - DNA, 19 bp, synthetic construct
  source 1..19: mol_type = other DNA
caggcatgagccactgtgc

SEQ ID NO: 21 - DNA, 29 bp, synthetic construct
  source 1..29: mol_type = other DNA
aaatgagatcaatcagtacacgatatctg

SEQ ID NO: 22 - DNA, 32 bp, synthetic construct
  source 1..32: mol_type = other DNA
cctccttattagaatctgtacttcactgtatt

SEQ ID NO: 23 - DNA, 33 bp, synthetic construct
  source 1..33: mol_type = other DNA
tttagtgggattgtttgttgtgcattctgttcc

SEQ ID NO: 24 - DNA, 29 bp, synthetic construct
  source 1..29: mol_type = other DNA
tttagtgggattgtttgtaaagctgggcg

SEQ ID NO: 25 - DNA, 19 bp, synthetic construct
  source 1..19: mol_type = other DNA
tgcttgaggccagcagttc

SEQ ID NO: 26 - DNA, 22 bp, synthetic construct
  source 1..22: mol_type = other DNA
accatgcctggctaacttcttc

SEQ ID NO: 27 - DNA, 19 bp, synthetic construct
  source 1..19: mol_type = other DNA
tgcttgaggccagcagttc

SEQ ID NO: 28 - DNA, 22 bp, synthetic construct
  source 1..22: mol_type = other DNA
ttgaggagagtggttttcgtga

SEQ ID NO: 29 - DNA, 33 bp, synthetic construct
  source 1..33: mol_type = other DNA
tgggcaacatagcaagaccctgtctttatttaa

SEQ ID NO: 30 - DNA, 30 bp, synthetic construct
  source 1..30: mol_type = other DNA
agcctgggcaacatagcaagagcttttaac